European Patent Application EP 4 653 461 A1, published November 26, 2025. Title: Novel Anti-NKp46 Antibodies and Use Thereof. Applicant: De novo Biotherapeutics. Application KR. The sequence listing filed with the application follows.

SEQUENCE LISTING (71 sequences)

SEQ ID NO: 1 - protein, 11 aa, synthetic construct
RTNENIFSYLA

SEQ ID NO: 2 - protein, 11 aa, synthetic construct
KASQSVSNDVA

SEQ ID NO: 3 - protein, 10 aa, synthetic construct
SASSSVGYMF

SEQ ID NO: 4 - protein, 11 aa, synthetic construct
KASQDINSYLS

SEQ ID NO: 5 - protein, 11 aa, synthetic construct
RASQDIGSSLN

SEQ ID NO: 6 - protein, 11 aa, synthetic construct
RASQDIGNSLN

SEQ ID NO: 7 - protein, 7 aa, synthetic construct
NAKTLAE

SEQ ID NO: 8 - protein, 7 aa, synthetic construct
YASNRYT

SEQ ID NO: 9 - protein, 7 aa, synthetic construct
RTSNLAS

SEQ ID NO: 10 - protein, 7 aa, synthetic construct
RANRLVD

SEQ ID NO: 11 - protein, 7 aa, synthetic construct
ATSSLDS

SEQ ID NO: 12 - protein, 7 aa, synthetic construct
ATSSLDA

SEQ ID NO: 13 - protein, 9 aa, synthetic construct
QHHYGTPYT

SEQ ID NO: 14 - protein, 9 aa, synthetic construct
HQDYSSPFT

SEQ ID NO: 15 - protein, 11 aa, synthetic construct
QQYHSYPPMWT

SEQ ID NO: 16 - protein, 9 aa, synthetic construct
LQYDEFPYT

SEQ ID NO: 17 - protein, 9 aa, synthetic construct
LQYASSPFT

SEQ ID NO: 18 - protein, 9 aa, synthetic construct
LQYASSPWT

SEQ ID NO: 19 - protein, 9 aa, synthetic construct
LQYDEFPWT

SEQ ID NO: 20 - protein, 107 aa, synthetic construct
DIQMTQSPASLSASVGETVTITCRTNENIFSYLAWYQQKQGKSPQLLVYNAKTLAEGVPSRFSGSASGTQFSLKINTLQPEDFGSYYCQHHYGTPYTFGGGTKLEII

SEQ ID NO: 21 - protein, 107 aa, synthetic construct
SIVMTQSPKFLLVSAGDRVTITCKASQSVSNDVAWYQQKPGQSPKLLIYYASNRYTGVPDRFTGSGYGTDFTFTISTVQAEDLAVYFCHQDYSSPFTFGSGTKLEIK

SEQ ID NO: 22 - protein, 108 aa, synthetic construct
QIVLTQSPAIMSASPGEKVTISCSASSSVGYMFWYQQKPGSSPKPWIYRTSNLASGVPARFSGSGSGTSYSLTISSMEAEDAATYYCQQYHSYPPMWTFGGGTKLEIK

SEQ ID NO: 23 - protein, 107 aa, synthetic construct
DIKMTQSPSSMYASLGERVTITCKASQDINSYLSWFQQKPGKSPKTLIYRANRLVDGVPSRFSGSGSGQDYSLTISSLEYEDVGMYYCLQYDEFPYTFGGGTKLEIK

SEQ ID NO: 24 - protein, 107 aa, synthetic construct
DIQMTQSPSSLSASLGERVSLTCRASQDIGSSLNWLQQEPDGTIKRLIYATSSLDSGVPKRFSGSRSGSDYSLTISSLESEDFVDYYCLQYASSPFTFGSGTKLEIK

SEQ ID NO: 25 - protein, 107 aa, synthetic construct
DIQMTQSPSSLSASLGERVSLTCRASQDIGSSLNWLQQEPDGTIKRLIYATSSLDSGVPKRFSGSRSGSDYSLTISSLESEDFVDYYCLQYASSPWTFGGGTKLEIK

SEQ ID NO: 26 - protein, 107 aa, synthetic construct
DIQMTQSPSSLSASLGERVTLTCRASQDIGSSLNWLQQEPDGTIKRLIYATSSLDSGVPKRFSGSRSGSDYSLTISSLESEDFVDYYCLQYASSPFTFGSGTKLEIK

SEQ ID NO: 27 - protein, 107 aa, synthetic construct
DIKMTQSPSSMYASLGERVTITCKASQDINSYLSWFQQKPGKSPKTLIYRANRLVDGVPSRFSGSGSGQDYSLTISSLEFEDLGIYYCLQYDEFPWTFGGGTKLEIK

SEQ ID NO: 28 - protein, 107 aa, synthetic construct; identical to SEQ ID NO: 24

SEQ ID NO: 29 - protein, 107 aa, synthetic construct
DIQMTQSPSSLSASLGERVSLTCRASQDIGNSLNWLQQEPDGTIKRLIYATSSLDSGVPKRFSGSRSGSDYSLTISSLESEDFVDYYCLQYASSPWTFGGGTKLEIK

SEQ ID NO: 30 - protein, 107 aa, synthetic construct
DIQMTQSPSSLSASVGDRVTITCRTNENIFSYLAWYQQKPGKAPKLLIYNAKTLAEGVPSRFSGSGSGTDFTLTISSLQPEDFATYYCQHHYGTPYTFGGGTKLEIK

SEQ ID NO: 31 - protein, 107 aa, synthetic construct
DIQMTQSPSSLSASVGDRVTITCRASQDIGSSLNWLQQKPGKAPKRLIYATSSLDAGVPKRFSGSGSGTDYTLTISSLQPEDFATYYCLQYASSPFTFGGGTKLEIK

SEQ ID NO: 32 - protein, 107 aa, synthetic construct
DIQMTQSPSSLSASVGDRVTITCKASQDINSYLSWFQQKPGKAPKSLIYRANRLVDGVPSRFSGSGSGTDYTLTISSLQPEDFATYYCLQYDEFPWTFGGGTKLEIK

SEQ ID NO: 33 - protein, 5 aa, synthetic construct
DYYLN

SEQ ID NO: 34 - protein, 5 aa, synthetic construct
NTYMH

SEQ ID NO: 35 - protein, 5 aa, synthetic construct
SYWMH

SEQ ID NO: 36 - protein, 5 aa, synthetic construct
SYWMN

SEQ ID NO: 37 - protein, 6 aa, synthetic construct
SDDYWN

SEQ ID NO: 38 - protein, 5 aa, synthetic construct
NYWMH

SEQ ID NO: 39 - protein, 17 aa, synthetic construct
DIDPHNGGTSYNQKFKD

SEQ ID NO: 40 - protein, 17 aa, synthetic construct
MIDPANGNTKYAPKFQG

SEQ ID NO: 41 - protein, 17 aa, synthetic construct
VIDPSDSYTNYNQKFKG

SEQ ID NO: 42 - protein, 17 aa, synthetic construct
MIHPNSGSTNYNEKFKS

SEQ ID NO: 43 - protein, 17 aa, synthetic construct
MIHPNSGVTKYNEKFKS

SEQ ID NO: 44 - protein, 17 aa, synthetic construct
MIHPNSDITNYNEKFKS

SEQ ID NO: 45 - protein, 16 aa, synthetic construct
YISYDGSNNYNPSLKN

SEQ ID NO: 46 - protein, 17 aa, synthetic construct
DIDPHNAGTSYNQKFKD

SEQ ID NO: 47 - protein, 16 aa, synthetic construct
YISYEGSNNYNPSLKN

SEQ ID NO: 48 - protein, 13 aa, synthetic construct
FPIYYSGSSPMDY

SEQ ID NO: 49 - protein, 13 aa, synthetic construct
WAYDGYYESYFDY

SEQ ID NO: 50 - protein, 12 aa, synthetic construct
SSSAYYSNYEAY

SEQ ID NO: 51 - protein, 11 aa, synthetic construct
EGNWARGYFEY

SEQ ID NO: 52 - protein, 6 aa, synthetic construct
DGRFAY

SEQ ID NO: 53 - protein, 6 aa, synthetic construct
HGRFDY

SEQ ID NO: 54 - protein, 8 aa, synthetic construct
LGYPAMDS

SEQ ID NO: 55 - protein, 6 aa, synthetic construct
GGRLDY

SEQ ID NO: 56 - protein, 8 aa, synthetic construct
LGYPAMDA

SEQ ID NO: 57 - protein, 122 aa, synthetic construct
EVQLQQSGPELVKPGASVKISCQASGYTFTDYYLNWVKQSHGKSLEWIGDIDPHNGGTSYNQKFKDKATLTVDKSSSTAYMELRSLTSEDSAVYYCARFPIYYSGSSPMDYWGQGTSVTVSS

SEQ ID NO: 58 - protein, 122 aa, synthetic construct
DVQLQQSVAELVRPGASVNLSCTASGFNIKNTYMHWVKQRPEQGLEWIGMIDPANGNTKYAPKFQGKATITADTSSNTAYLHLSSLTSEDTAIYYCARWAYDGYYESYFDYWGQGTTLTVSS

SEQ ID NO: 59 - protein, 121 aa, synthetic construct
QVQLQQPGAELVRPGTSVKLSCKASGYTFTSYWMHWVKQRPGQGLEWIGVIDPSDSYTNYNQKFKGKATLTVDTSSSTAYMQLSSLTSEDSAVYYCARSSSAYYSNYEAYWGQGTLVTVSA

SEQ ID NO: 60 - protein, 120 aa, synthetic construct
QVQLQQPGAELVKPGASVKLSCKASGYIFTSYWMHWVKQRPGQGLEWIGMIHPNSGSTNYNEKFKSKATLTVDKSSSTAYMQLSSLTSEDSAVYYCAREGNWARGYFEYWGQGTTLTVSS

SEQ ID NO: 61 - protein, 115 aa, synthetic construct
QVQLQQPGAELVKPGASVKLSCKASGYTFTSYWMHWVKQRPGQGLEWIGMIHPNSGSTNYNEKFKSKATLTVDKSSSTAYMQLSSLTSEDSAVYYCVYDGRFAYWGQGTLVTVSA

SEQ ID NO: 62 - protein, 115 aa, synthetic construct
QVQLQQPGAELVKPGASVKLSCKASGYTFTSYWMHWVKQRPGQGLEWIGMIHPNSGVTKYNEKFKSKATLTVDKSSSTAYMQLSSLTSEDSAVYFCAGDGRFAYWGQGTLVTVSA

SEQ ID NO: 63 - protein, 115 aa, synthetic construct
QVQLQQPGAELVKPGASVKLSCKASGYTFTSYWMNWVKQRPGQGLEWIGMIHPNSDITNYNEKFKSQATLTVDKSSSTAYMQLSSLTSEDSAVYYCARHGRFDYWGQGTTLTVSS

SEQ ID NO: 64 - protein, 117 aa, synthetic construct
DVQLQESGPGLVKTSQSLSLTCSVTGYSITSDDYWNWIRQFPGNKLEWVGYISYDGSNNYNPSLKNRISITRDTSKNQFFLKLNSVTTEDTATYYCARLGYPAMDSWGQGTSVTVSS

SEQ ID NO: 65 - protein, 115 aa, synthetic construct
QVQLQQPGAELVKPGASVKLSCKASGFTFTNYWMHWVKQRPGQGLEWIGMIHPNSGSTNYNEKFKSKATLTVDKSSSTAYMQLSSLTSEDSAVYYCAGGGRLDYWGQGTTLTVSS

SEQ ID NO: 66 - protein, 115 aa, synthetic construct
QVQLQQPGAELVKPGASVRLSCKAFGYTFTSYWMHWVKQRPGQGLEWIGMIHPNSGVTKYNEKFKSKATLTVDKSSSTAYMQLSSLTSEDSAVYFCAGDGRFAYWGQGTLVTVSA

SEQ ID NO: 67 - protein, 122 aa, synthetic construct
QVQLVQSGAEVKKPGASVKVSCKASGYTFTDYYLNWVRQAPGQGLEWIGDIDPHNAGTSYNQKFKDRVTMTVDTSTSTVYMELSSLRSEDTAVYYCARFPIYYSGSSPMDYWGQGTLVTVSS

SEQ ID NO: 68 - protein, 115 aa, synthetic construct
QVQLVQSGAEVKKPGASVKVSCKASGYTFTSYWMNWVRQAPGQGLEWIGMIHPNSDITNYNEKFKSRVTMTVDTSTSTVYMELSSLRSEDTAVYYCARHGRFDYWGQGTTVTVSS

SEQ ID NO: 69 - protein, 117 aa, synthetic construct
QVQLQESGPGLVKPSQTLSLTCTVSGYSITSDDYWNWIRQPPGKGLEWIGYISYEGSNNYNPSLKNRVTISRDTSKNQFSLKLSSVTAADTAVYYCARLGYPAMDAWGQGTLVTVSS

SEQ ID NO: 70 - protein, 327 aa, synthetic construct
ASTKGPSVFPLAPCSRSTSESTAALGCLVKDYFPEPVTVSWNSGALTSGVHTFPAVLQSSGLYSLSSVVTVPSSSLGTKTYTCNVDHKPSNTKVDKRVESKYGPPCPPCPAPEFLGGPSVFLFPPKPKDTLMISRTPEVTCVVVDVSQEDPEVQFNWYVDGVEVHNAKTKPREEQFNSTYRVVSVLTVLHQDWLNGKEYKCKVSNKGLPSSIEKTISKAKGQPREPQVYTLPPSQEEMTKNQVSLTCLVKGFYPSDIAVEWESNGQPENNYKTTPPVLDSDGSFFLYSRLTVDKSRWQEGNVFSCSVMHEALHNHYTQKSLSLSLGK

SEQ ID NO: 71 - protein, 107 aa, synthetic construct [sequence omitted]